European Patent Specification EP 3 652 336 B1, published April 17, 2024. Title: METHOD FOR DETECTING A MUTATION IN A MICROSATELLITE SEQUENCE. Applicant: Institut Curie Université Versailles Saint-Quentin-En-Yvelines INSERM. The sequence listing filed with the application follows.

SEQUENCE LISTING (20 sequences)

SEQ ID NO: 1 - DNA, 31 bp, Artificial Sequence
  primer
gacttcagccagtatatgaaattggatattg

SEQ ID NO: 2 - DNA, 36 bp, Artificial Sequence
  primer
gtatatgtcaatgaaaacattttttaaccattcaac

SEQ ID NO: 3 - DNA, 23 bp, Artificial Sequence
  Probe
agcagtcagagcccttaaccttt

SEQ ID NO: 4 - DNA, 33 bp, Artificial Sequence
  Probe
aggtaaaaaaaaaaaaaaaaaaaaaaaaaaagg

SEQ ID NO: 5 - DNA, 22 bp, Artificial Sequence
  Primer
gaggaggaaattggccagcatc

SEQ ID NO: 6 - DNA, 25 bp, Artificial Sequence
  Primer
agctaactggataacttacagcatg

SEQ ID NO: 7 - DNA, 22 bp, Artificial Sequence
  Probe
acttcctgcatgtcttcaagag

SEQ ID NO: 8 - DNA, 16 bp, artificial sequence
  Probe
cctcttttttttatgc

SEQ ID NO: 9 - DNA, 25 bp, artificial sequence
  Primer
ttgaaaaatctgggctgattcttga

SEQ ID NO: 10 - DNA, 22 bp, artificial sequence
  Primer
tgagggagctttccaggaaatg

SEQ ID NO: 11 - DNA, 24 bp, artificial sequence
  Probe
ctttgacatgttccccatttctag

SEQ ID NO: 12 - DNA, 16 bp, artificial sequence
  Probe
tccctttttttttggt

SEQ ID NO: 13 - DNA, 27 bp, artificial sequence
  Primer
tgaagacctcacagtaaaaataggtga

SEQ ID NO: 14 - DNA, 21 bp, artificial sequence
  Primer
actgatgggacccactccatc

SEQ ID NO: 15 - DNA, 15 bp, artificial sequence
  Probe
tagctacagtgaaat

SEQ ID NO: 16 - DNA, 16 bp, artificial sequence
  Probe
ctagctacagagaaat

SEQ ID NO: 17 - DNA, 24 bp, artificial sequence
  Primer
cagcatgtttctgccaataatctc

SEQ ID NO: 18 - DNA, 18 bp, artificial sequence
  Probe
aggcctcttttttttatg

SEQ ID NO: 19 - DNA, 20 bp, artificial sequence
  Primer
gccaagaaagagctgctgag

SEQ ID NO: 20 - DNA, 21 bp, artificial sequence
  Probe
aactgtccctttttttttggt